European Patent Application EP 4 194 563 A1, published June 14, 2023. Title: TRANSPOSASE COMPETITOR CONTROL SYSTEM. Applicant: KAPA BIOSYSTEMS, INC. Application EP. The sequence listing filed with the application follows.

SEQUENCE LISTING (58 sequences)

SEQ ID NO: 1 - protein, 476 aa, synthetic construct
MITSALHRAADWAKSVFSSAALGDPRRTARLVNVAAQLAKYSGKSITISSEGSKAAQEGAYRFIRNPNVSAEAIRKAGAMQTVKLAQEFPELLAIEDTTSLSYRHQVAEELGKLGSIQDKSRGWWVHSVLLLEATTFRTVGLLHQEWWMRPDDPADADEKESGKWLAAAATSRLRMGSMMSNVIAVCDREADIHAYLQDKLAHNERFVVRSKHPRKDVESGLYLYDHLKNQPELGGYQISIPQKGVVDKRGKRKNRPARKASLSLRSGRITLKQGNITLNAVLAEEINPPKGETPLKWLLLTSEPVESLAQALRVIDIYTHRWRIEEFHKAWKTGAGAERQRMEEPDNLERMVSILSFVAVRLLQLRESFTPPQALRAQGLLKEAEHVESQSAETVLTPDECQLLGYLDKGKRKRKEKAGSLQWAYMAIARLGGFMDSKRTGIASWGALWEGWEALQSKLDGFLAAKDLMAQGIKI

SEQ ID NO: 2 - protein, 455 aa, synthetic construct
MNNAQWAKSTFGQADLGDPRRTTRLVKLAETLANDPGKPFVSITQSPADMEGAYRFIRNEHVNADAIAKAGYLVTAAQAAKHNLLLALEDTTAITYSHRSVRDELGHVNQGNNYRGILAHSVLLFAPEQQELVGLIEQSRWTRDISTRGKKHVRTQTPYEEKESFKWQSASVNLSARLGTKMADVISVCDREADIYEYLQYKLSKQHRFVVRSMQSRHIEQSEQKLYDYAAGLESAGQKQIHIAQKGGRKARTATVDIVFAPVTLQVPANKRGESLSLYYVGCEERADDKNALNWHLLTTEPVQSKADALNIIRYYEHRWLVEEYHKAWKTDGTDIENARLQSKDNIERLVTISAFIAVRIVQLKFAREQPDEISCEQVLSPKAWKLLWIKRVSRTLPDTVPSMKWAYTELAKLGGWKDTKQTGKASVKVLWQGWFKLQTILEGYDLAKSLEADL

SEQ ID NO: 3 - protein, 455 aa, synthetic construct; identical to SEQ ID NO: 2

SEQ ID NO: 4 - protein, 476 aa, synthetic construct
MITSALHRAADWAKSVFSSAALGDPRRTARLVNVAAQLAKYSGKSITISSEGSKAAQEGAYRFIRNPNVSAEAIRKAGAMQTVKLAQEFPELLAIEDTTSLSYRHQVAEELGKLGSIQDKSRGWWVHSVLLLEATTFRTVGLLHQEWWMRPDDPADADEKESGMWLAAAATSRLRMGSMMSNVIAVCDREADIHAYLQDKLAHNERFVVRSKHPRKDVESGLYLYDHLKNQPELGGYQISIPQKGVVDKRGKRKNRPARKASLSLRSGRITLKQGNITLNAVLAEEINPPKGETPLKWLLLTSEPVESLAQALRVIDIYTHRWRIEEFHKAWKTGAGAERQRMEEPDNLERMVSILSFVAVRLLQLRESFTPPQALRAQGLLKEAEHVESQSAETVLTPDECQLLGYLDKGKRKRKEKAGSLQWAYMAIARLGGFMDSKRTGIASWGALWEGWEALQSKLDGFLAAKDLMAQGIKI

SEQ ID NO: 5 - DNA, 19 bp, synthetic construct
  source 1..19: mol_type = other DNA
agatgtgtataagagacag

SEQ ID NO: 6 - DNA, 19 bp, synthetic construct
  source 1..19: mol_type = other DNA
tctacacatattctctgtc

SEQ ID NO: 7 - DNA, 19 bp, synthetic construct
  modified_base 19: mod_base = OTHER; note = modification may include 3'-H, 3'-phosphate, 3'-bulky group selected from the group consisting of a hexanediol, a 3-carbon spacer, a triethylene glycol, a hexa-ethyleneglycol, and any combination thereof
  source 1..19: mol_type = other DNA
agatgtgtataagagacag

SEQ ID NO: 8 - DNA, 19 bp, synthetic construct
  source 1..19: mol_type = other DNA
tctacacatattctctgtc

SEQ ID NO: 9 - DNA, 19 bp, synthetic construct
  modified_base 19: mod_base = OTHER; note = modification is a 3'-H
  source 1..19: mol_type = other DNA
agatgtgtataagagacag

SEQ ID NO: 10 - DNA, 19 bp, synthetic construct
  source 1..19: mol_type = other DNA
tctacacatattctctgtc

SEQ ID NO: 11 - DNA, 19 bp, synthetic construct
  modified_base 19: mod_base = OTHER; note = modification is a 3'-phosphate
  source 1..19: mol_type = other DNA
agatgtgtataagagacag

SEQ ID NO: 12 - DNA, 19 bp, synthetic construct
  source 1..19: mol_type = other DNA
tctacacatattctctgtc

SEQ ID NO: 13 - DNA, 19 bp, synthetic construct
  modified_base 19: mod_base = OTHER; note = N may include a synthetic base, a nucleotide analog (e.g. alocked nucleic acid, a bridged nucleic acid, or a xeno nucleicacid), an inverted base, or an abasic site.
  source 1..19: mol_type = other DNA
agatgtgtataagagacan

SEQ ID NO: 14 - DNA, 19 bp, synthetic construct
  source 1..19: mol_type = other DNA
tctacacatattctctgtc

SEQ ID NO: 15 - protein, 476 aa, synthetic construct; identical to SEQ ID NO: 1

SEQ ID NO: 16 - protein, 455 aa, synthetic construct; identical to SEQ ID NO: 2

SEQ ID NO: 17 - protein, 461 aa, synthetic construct
MTYIEPTLWAQKQFGQAHLNDPRRTQRLVALAASLAEQPGVPVSKLIISPADMEGAYRFIRNEQIKAEDIAEAGFHVTAQEALEQQTLLALEDTTSLSYSHRSIQDELGHSNQGNRNRAMFIHSTLLFAPETQVVVGLIEQQRWTRDIEKRGQGHQYATRPYKEKESYKWEQASRHVAERLGDKISDVISVCDREADLFEYLTYKQEQQQRFLVRSMQSRCIEEHDNRLYDYASKLQSAGERVLDIPQKGGRKARTVHLDIKYAPVTLKSPANKKEFNNIPLYYVGCIEQGESNDKLAWHLLTSEPITSKEEALKIVSYYELRWLIEDFHKVWKSEGTQVEQLRMQSKDNLERLSVILAFIATRLLQLRFMNESDELSKSSCEPILKGKAWKLMWLKLERKGLPKEAPDISWAYKGIARLGGWKNTKRTGRASIKTLWQGWFRLQTILEGYELAKSLDSPD

SEQ ID NO: 18 - protein, 459 aa, synthetic construct
MTHSDAKLWAQEQFGQAQLKDPRRTQRLISLATSIANQPGVSVAKLPFSPADMEGAYRFIRNENINAEDIAEAGFQSTVSRANEHKELLALEDTTTLSFPHRSIKEELGHTNQGDRTRALHVHSTLLFAPQSQTIVGLIEQQRWSRDITKRGQKHQHATRPYKEKESYKWEQASRRVVERLGDKMLDVISVCDREADLFEYLTYKRQHQQRFVVRSMQSRCLEEHAQKLYDYAQALPSVETKALTIPQKGGRKARNVKLDVKYGQVTLKAPANKKEHAGIPVYYVGCLEQGTSKDKLAWHLLTSEPINNVDDAMRIIGYYERRWLIEDFHKVWKSEGTDVESLRLQSKDNLERLSVIYAFVATRLLALRFMKEVDELTKESCEKVLGQKAWKLLWLKLESKTLPKEVPDMGWAYKNLAKLGGWKDTKRTGRASIKVLWEGWFKLQTILEGYELAMSLDH

SEQ ID NO: 19 - protein, 457 aa, synthetic construct
MIKSNNDWAEEQFGHAKLGDPRRTARLVKMASDLAQHPGKSVVKSSPSPASMEGAYRFIRNDNVSADDIAEAGFRATVNQAHRYPLLLAIEDTTTLSYKHRSIRADLGHVNQGNRYRGLLAHSILLFAPETLDVVGLIEQHRWTRDIKTRGIRRENLKRPYEEKEGYKWESASRNMAARLGTAMANVISVCDREADIYDYLLYKIANQQRFVVRSMMSRHIEEGSDKLYHFASELNSVKQRQIQIAQRGGRKAREVTLDVKYAAVTLKTPANKKGSPISLNYVGCSEVGDEEKTLNWHILTNEPVNSAEDALKIIGYYEKRWLIEEYHKVWKSEGTGVEDLRVQSKDNLDRLATIYAFLAVRIFQLKFANEQIEDISSEKILSPRAWKLLWLKRIKTPPPEEVPTAKWAYEHLARLGGWKDSKRNGRASVKTLWEGWLKLQAILEGYELALSLEQDL

SEQ ID NO: 20 - protein, 342 aa, synthetic construct
MITSALHRAADWAKSVFSSAALGDPRRTARLVNVAAQLAKYSGKSITISSEGSEAMQEGAYRFIRNPNVSAEAIRKAGAMQTVKLAQEFPELLAIEDTTSLSYRHQVAEELGKLGSIQDKSRGWWVHSVLLLEATTFRTVGLLHQEWWMRPDDPADADEKESGKWLAAAATSRLRMGSMMSNVIAVCDREADIHAYLQDKLAHNERFVVRSKHPRKDVESGLYLYDHLKNQPELGGYQISIPQKGVVDKRGKRKNRPARKASLSLRSGRITLKQGNITLNAVLAEEINPPKGETPLKWLLLTSEPVESLAQALRVIDIYTHRWRIEEFHKAWKTGAGAERQR

SEQ ID NO: 21 - protein, 342 aa, synthetic construct
MITSALHRAADWAKSVFSSAALGDPRRTARLVNVAAQLAKYSGKSITISSEGSKAAQEGAYRFIRNPNVSAEAIRKAGAMQTVKLAQEFPELLAIEDTTSLSYRHQVAEELGKLGSIQDKSRGWWVHSVLLLEATTFRTVGLLHQEWWMRPDDPADADEKESGKWLAAAATSRLRMGSMMSNVIAVCDREADIHAYLQDKLAHNERFVVRSKHPRKDVESGLYLYDHLKNQPELGGYQISIPQKGVVDKRGKRKNRPARKASLSLRSGRITLKQGNITLNAVLAEEINPPKGETPLKWLLLTSEPVESLAQALRVIDIYTHRWRIEEFHKAWKTGAGAERQR

SEQ ID NO: 22 - protein, 340 aa, synthetic construct
MNNAQWAKSTFGQADLGDPRRTTRLVKLAETLANDPGKPFVSITQSPADMEGAYRFIRNEHVNADAIAKAGYLVTAAQAAKHNLLLALEDTTAITYSHRSVRDELGHVNQGNNYRGILAHSVLLFAPEQQELVGLIEQSRWTRDISTRGKKHVRTQTPYEEKESFKWQSASVNLSARLGTKMADVISVCDREADIYEYLQYKLSKQHRFVVRSMQSRHIEQSEQKLYDYAAGLESAGQKQIHIAQKGGRKARTATVDIVFAPVTLQVPANKRGESLSLYYVGCEERADDKNALNWHLLTTEPVQSKADALNIIRYYEHRWLVEEYHKAWKTDGTDIENAR

SEQ ID NO: 23 - protein, 342 aa, synthetic construct
MIKSNNDWAEEQFGHAKLGDPRRTARLVKMASDLAQHPGKSVVKSSPSPASMEGAYRFIRNDNVSADDIAEAGFRATVNQAHRYPLLLAIEDTTTLSYKHRSIRADLGHVNQGNRYRGLLAHSILLFAPETLDVVGLIEQHRWTRDIKTRGIRRENLKRPYEEKEGYKWESASRNMAARLGTAMANVISVCDREADIYDYLLYKIANQQRFVVRSMMSRHIEEGSDKLYHFASELNSVKQRQIQIAQRGGRKAREVTLDVKYAAVTLKTPANKKGSPISLNYVGCSEVGDEEKTLNWHILTNEPVNSAEDALKIIGYYEKRWLIEEYHKVWKSEGTGVEDLR

SEQ ID NO: 24 - protein, 344 aa, synthetic construct
MTYIEPTLWAQKQFGQAHLNDPRRTQRLVALAASLAEQPGVPVSKLIISPADMEGAYRFIRNEQIKAEDIAEAGFHVTAQEALEQQTLLALEDTTSLSYSHRSIQDELGHSNQGNRNRAMFIHSTLLFAPETQVVVGLIEQQRWTRDIEKRGQGHQYATRPYKEKESYKWEQASRHVAERLGDKISDVISVCDREADLFEYLTYKQEQQQRFLVRSMQSRCIEEHDNRLYDYASKLQSAGERVLDIPQKGGRKARTVHLDIKYAPVTLKSPANKKEFNNIPLYYVGCIEQGESNDKLAWHLLTSEPITSKEEALKIVSYYELRWLIEDFHKVWKSEGTQVEQLR

SEQ ID NO: 25 - protein, 344 aa, synthetic construct
MTHSDAKLWAQEQFGQAQLKDPRRTQRLISLATSIANQPGVSVAKLPFSPADMEGAYRFIRNENINAEDIAEAGFQSTVSRANEHKELLALEDTTTLSFPHRSIKEELGHTNQGDRTRALHVHSTLLFAPQSQTIVGLIEQQRWSRDITKRGQKHQHATRPYKEKESYKWEQASRRVVERLGDKMLDVISVCDREADLFEYLTYKRQHQQRFVVRSMQSRCLEEHAQKLYDYAQALPSVETKALTIPQKGGRKARNVKLDVKYGQVTLKAPANKKEHAGIPVYYVGCLEQGTSKDKLAWHLLTSEPINNVDDAMRIIGYYERRWLIEDFHKVWKSEGTDVESLR

SEQ ID NO: 26 - protein, 134 aa, synthetic construct
MEEPDNLERMVSILSFVAVRLLQLRESFTLPQALRAQGLLKEAEHVESQSAETVLTPDECQLLGYLDKGKRKRKEKAGSLQWAYMAIARLGGFMDSKRTGIASWGALWEGWEALQSKLDGFLAAKDLMAQGIKI

SEQ ID NO: 27 - protein, 134 aa, synthetic construct
MEEPDNLERMVSILSFVAVRLLQLRESFTPPQALRAQGLLKEAEHVESQSAETVLTPDECQLLGYLDKGKRKRKEKAGSLQWAYMAIARLGGFMDSKRTGIASWGALWEGWEALQSKLDGFLAAKDLMAQGIKI

SEQ ID NO: 28 - protein, 115 aa, synthetic construct
LQSKDNIERLVTISAFIAVRIVQLKFAREQPDEISCEQVLSPKAWKLLWIKRVSRTLPDTVPSMKWAYTELAKLGGWKDTKQTGKASVKVLWQGWFKLQTILEGYDLAKSLEADL

SEQ ID NO: 29 - protein, 115 aa, synthetic construct
VQSKDNLDRLATIYAFLAVRIFQLKFANEQIEDISSEKILSPRAWKLLWLKRIKTPPPEEVPTAKWAYEHLARLGGWKDSKRNGRASVKTLWEGWLKLQAILEGYELALSLEQDL

SEQ ID NO: 30 - protein, 117 aa, synthetic construct
MQSKDNLERLSVILAFIATRLLQLRFMNESDELSKSSCEPILKGKAWKLMWLKLERKGLPKEAPDISWAYKGIARLGGWKNTKRTGRASIKTLWQGWFRLQTILEGYELAKSLDSPD

SEQ ID NO: 31 - protein, 115 aa, synthetic construct
LQSKDNLERLSVIYAFVATRLLALRFMKEVDELTKESCEKVLGQKAWKLLWLKLESKTLPKEVPDMGWAYKNLAKLGGWKDTKRTGRASIKVLWEGWFKLQTILEGYELAMSLDH

SEQ ID NO: 32 - protein, 455 aa, synthetic construct
MNNAQWAKSTFGQADLGDPRRTTRLVKLAETLANDPGKPFVSITQSKADMEGAYRFIRNEHVNADAIAKAGYLVTAAQAAKHNLLLALEDTTAITYSHRSVRDELGHVNQGNNYRGILAHSVLLFAPEQQELVGLIEQSRWTRDISTRGKKHVRTQTPYEEKESFKWQSASVNLSARLGTKMADVISVCDREADIYEYLQYKLSKQHRFVVRSMQSRHIEQSEQKLYDYAAGLESAGQKQIHIAQKGGRKARTATVDIVFAPVTLQVPANKRGESLSLYYVGCEERADDKNALNWHLLTTEPVQSKADALNIIRYYEHRWLVEEYHKAWKTDGTDIENARLQSKDNIERLVTISAFIAVRIVQLKFAREQPDEISCEQVLSPKAWKLLWIKRVSRTLPDTVPSMKWAYTELAKLGGWKDTKQTGKASVKVLWQGWFKLQTILEGYDLAKSLEADL

SEQ ID NO: 33 - protein, 455 aa, synthetic construct
MNNAQWAKSTFGQADLGDPRRTTRLVKLAETLANDPGKPFVSITQSPADAEGAYRFIRNEHVNADAIAKAGYLVTAAQAAKHNLLLALEDTTAITYSHRSVRDELGHVNQGNNYRGILAHSVLLFAPEQQELVGLIEQSRWTRDISTRGKKHVRTQTPYEEKESFKWQSASVNLSARLGTKMADVISVCDREADIYEYLQYKLSKQHRFVVRSMQSRHIEQSEQKLYDYAAGLESAGQKQIHIAQKGGRKARTATVDIVFAPVTLQVPANKRGESLSLYYVGCEERADDKNALNWHLLTTEPVQSKADALNIIRYYEHRWLVEEYHKAWKTDGTDIENARLQSKDNIERLVTISAFIAVRIVQLKFAREQPDEISCEQVLSPKAWKLLWIKRVSRTLPDTVPSMKWAYTELAKLGGWKDTKQTGKASVKVLWQGWFKLQTILEGYDLAKSLEADL

SEQ ID NO: 34 - protein, 455 aa, synthetic construct
MNNAQWAKSTFGQADLGDPRRTTRLVKLAETLANDPGKPFVSITQSKADAEGAYRFIRNEHVNADAIAKAGYLVTAAQAAKHNLLLALEDTTAITYSHRSVRDELGHVNQGNNYRGILAHSVLLFAPEQQELVGLIEQSRWTRDISTRGKKHVRTQTPYEEKESFKWQSASVNLSARLGTKMADVISVCDREADIYEYLQYKLSKQHRFVVRSMQSRHIEQSEQKLYDYAAGLESAGQKQIHIAQKGGRKARTATVDIVFAPVTLQVPANKRGESLSLYYVGCEERADDKNALNWHLLTTEPVQSKADALNIIRYYEHRWLVEEYHKAWKTDGTDIENARLQSKDNIERLVTISAFIAVRIVQLKFAREQPDEISCEQVLSPKAWKLLWIKRVSRTLPDTVPSMKWAYTELAKLGGWKDTKQTGKASVKVLWQGWFKLQTILEGYDLAKSLEADL

SEQ ID NO: 35 - DNA, 33 bp, synthetic construct
  source 1..33: mol_type = other DNA
tcgtcggcagcgtcagatgtgtataagagacag

SEQ ID NO: 36 - DNA, 19 bp, synthetic construct
  source 1..19: mol_type = other DNA
tctacacatattctctgtc

SEQ ID NO: 37 - DNA, 34 bp, synthetic construct
  source 1..34: mol_type = other DNA
gtctcgtgggctcggagatgtgtataagagacag

SEQ ID NO: 38 - DNA, 19 bp, synthetic construct
  source 1..19: mol_type = other DNA
tctacacatattctctgtc

SEQ ID NO: 39 - DNA, 33 bp, synthetic construct; identical to SEQ ID NO: 35
  source 1..33: mol_type = other DNA

SEQ ID NO: 40 - DNA, 19 bp, synthetic construct
  source 1..19: mol_type = other DNA
tctacacatattctctgtc

SEQ ID NO: 41 - DNA, 34 bp, synthetic construct; identical to SEQ ID NO: 37
  source 1..34: mol_type = other DNA

SEQ ID NO: 42 - DNA, 19 bp, synthetic construct
  source 1..19: mol_type = other DNA
tctacacatattctctgtc

SEQ ID NO: 43 - DNA, 33 bp, synthetic construct; identical to SEQ ID NO: 35
  source 1..33: mol_type = other DNA

SEQ ID NO: 44 - DNA, 19 bp, synthetic construct
  source 1..19: mol_type = other DNA
tctacacatattctctgtc

SEQ ID NO: 45 - DNA, 34 bp, synthetic construct; identical to SEQ ID NO: 37
  source 1..34: mol_type = other DNA

SEQ ID NO: 46 - DNA, 19 bp, synthetic construct
  source 1..19: mol_type = other DNA
tctacacatattctctgtc

SEQ ID NO: 47 - DNA, 19 bp, synthetic construct
  source 1..19: mol_type = other DNA
agatgtgtataagagacag

SEQ ID NO: 48 - DNA, 19 bp, synthetic construct
  source 1..19: mol_type = other DNA
tctacacatattctctgtc

SEQ ID NO: 49 - DNA, 33 bp, synthetic construct; identical to SEQ ID NO: 35
  source 1..33: mol_type = other DNA

SEQ ID NO: 50 - DNA, 19 bp, synthetic construct
  source 1..19: mol_type = other DNA
tctacacatattctctgtc

SEQ ID NO: 51 - DNA, 34 bp, synthetic construct; identical to SEQ ID NO: 37
  source 1..34: mol_type = other DNA

SEQ ID NO: 52 - DNA, 19 bp, synthetic construct
  source 1..19: mol_type = other DNA
tctacacatattctctgtc

SEQ ID NO: 53 - DNA, 19 bp, synthetic construct
  modified_base 19: mod_base = OTHER; note = modification is a 3'-phosphate
  source 1..19: mol_type = other DNA
agatgtgtataagagacag

SEQ ID NO: 54 - DNA, 19 bp, synthetic construct
  source 1..19: mol_type = other DNA
tctacacatattctctgtc

SEQ ID NO: 55 - DNA, 19 bp, synthetic construct
  misc_feature 19: note = 3'-spacer referred to as /"3SpC3"/
  source 1..19: mol_type = other DNA
agatgtgtataagagacag

SEQ ID NO: 56 - DNA, 19 bp, synthetic construct
  source 1..19: mol_type = other DNA
tctacacatattctctgtc

SEQ ID NO: 57 - DNA, 51 bp, synthetic construct
  misc_feature 50..51: note = phosphorothioate bond
  source 1..51: mol_type = other DNA
aatgatacggcgaccaccgagatctacactagatcgctcgtcggcagcgtc

SEQ ID NO: 58 - DNA, 47 bp, synthetic construct
  misc_feature 46..47: note = phosphorothioate bond
  source 1..47: mol_type = other DNA
caagcagaagacggcatacgagattcgccttagtctcgtgggctcgg